European Patent Specification EP 3 618 881 B1, published February 15, 2023. Title: Post-3D Printing Functionalization of Polymer Scaffolds For Enhanced Bioactivity. Applicant: The University of Akron. The sequence listing filed with the application follows.

SEQUENCE LISTING (16 sequences)

SEQ ID NO: 1 - protein, 8 aa, Artificial
  Artificially generated sequence for basic fibroblast growth factor
  misc_feature: bFGF (basic Fibroblast Growth Factor)
CYKRSRYT

SEQ ID NO: 2 - protein, 21 aa, Artificial
  Artificially generated sequence for Bone Morphogenic Protein 2
CKIPKASSVPTELSAISTLYL

SEQ ID NO: 3 - protein, 5 aa, Artificial
  Artificially generated sequence containing residues 10 through 14 of Osteogenic Growth Peptide  (OGP)
  misc_feature: Residues 10-14 of Osteogenic Growth Peptide (OGP)
YGFGG

SEQ ID NO: 4 - protein, 20 aa, Artificial
  Artificially generated sequence for Bone Morphogenic Protein 2 73-92
KIPKASSVPTELSAISTLYL

SEQ ID NO: 5 - protein, 20 aa, Artificial
  Artificially generated sequence for Bone Morphogenic Protein-7 89-117
TVPKPSSAPTQLNAISTLYF

SEQ ID NO: 6 - protein, 20 aa, Artificial
  Artificially generated sequence for Bone Morphogenic Protein-9 68-87
  misc_feature: BMP-9 68-87
KVGKASSVPTKLSPISILYK

SEQ ID NO: 7 - DNA, 18 bp, Artificial
  Artificially generated forward primer sequence for hGAPDH
  misc_feature: hGAPDH primer (forward sequence)
gacagtcagccgcatctt

SEQ ID NO: 8 - DNA, 20 bp, Artificial
  Artificially generated reverse primer sequence for hGAPDH
  misc_feature: hGAPDH primer (reverse sequence)
ccatggtgtctgagcgatgt

SEQ ID NO: 9 - DNA, 20 bp, Artificial
  Artificially generated forward primer sequence for hRunx2
  misc_feature: hRunx2 primer (forward sequence)
ggacgaggcaagagtttcac

SEQ ID NO: 10 - DNA, 26 bp, Artificial
  Artificially generated reverse primer sequence for hRunx2
  misc_feature: hRunx2 primer (reverse sequence)
artcacaagcttctgtctgtgccttc

SEQ ID NO: 11 - DNA, 20 bp, Artificial
  Artificially generated forward primer sequence for hBSP
  misc_feature: hBSP primer (forward sequence)
cctggcacagggtatacagg

SEQ ID NO: 12 - DNA, 20 bp, Artificial
  Artificially generated reverse primer sequence for hBSP
  misc_feature: hBSP primer (reverse sequence)
ctgcttcgctttcttcgttt

SEQ ID NO: 13 - DNA, 15 bp, Artificial
  Artificially generated forward primer sequence for hOCN
  misc_feature: hOCN primer (forward sequence)
catgagagccctcac

SEQ ID NO: 14 - DNA, 17 bp, Artificial
  Artificially generated reverse primer sequence for hOCN
  misc_feature: hOCN primer (reverse sequence)
agagcgacaccctagac

SEQ ID NO: 15 - DNA, 23 bp, Artificial
  Artificially generated forward primer sequence for hCD31
  misc_feature: hCD31 primer (forward sequence)
tctatgacctcgccctccacaaa

SEQ ID NO: 16 - DNA, 27 bp, Artificial
  Artificially generated reverse primer sequence for hCD31
  misc_feature: hCD31 primer (reverse sequence)
gaacggtgtcttcaggttggtatttca